European Patent Application EP 4 591 870 A1, published July 30, 2025. Title: An antibacterial composition and a method for determining the administration thereof to a subject. Applicant: JSR株式会社. The sequence listing filed with the application follows.

SEQUENCE LISTING (15 sequences)

SEQ ID NO: 1 - DNA, 313 bp, Actinomyces viscosus
  source 1..313: mol_type = genomic DNA
gacgaacgctggcggcgtgcttaacacatgcaagtcgaacggtgaaggagccagcttgctggttctggatgagtggcgaacgggtgagtaacacgtgagtaacctgcccccttcttctggataaccgcatgaaagtgtggctaatacgggatattctgggtctgtcgcatggtgggcctgggaaaggtttgttccggtgggggatgggctcgcggcctatcagcttgttggtggggtgatggcctaccaaggcggtgacgggtagccggcctgagagggtggacggtcacactgggactgagacacggcccag

SEQ ID NO: 2 - DNA, 304 bp, Cutibacterium granulosum
  source 1..304: mol_type = genomic DNA
gacgaacgctggcggcgtgcttaacacatgcaagtcgtacggtaaggccctttcgggggtacacgagtggcgaacgggtgagtaacacgtgagtaacctgcccacaactttgggataacgctaggaaactggtgctaatactggatatgtgctcctgctgcatggtgggggttggaaagctccggcggttgtggatggactcgcggcctatcagcttgttggtggggtagtggcctaccaaggcggcgacgggtagccggcctgagagggtgaccggccacattgggactgagatacggcccag

SEQ ID NO: 3 - DNA, 316 bp, Streptococcus oralis
  source 1..316: mol_type = genomic DNA
gacgaacgctggcggcgtgcctaatacatgcaagtagaacgctgaagcttggtgcttgcaccgagcggatgagttgcgaacgggtgagtaacgcgtaggtaacctgcctggtagcgggggataactattggaaacgatagctaataccgcataagagtagatgttgcatgacatttacttaaaaggtgcaattgcatcactaccagatggacctgcgttgtattagctagttggtgaggtaacggctcaccaaggcaacgatacatagccgacctgagagggtgatcggccacactgggactgagacacggcccag

SEQ ID NO: 4 - DNA, 317 bp, Staphylococcus warneri
  source 1..317: mol_type = genomic DNA
gatgaacgctggcggcgtgcctaatacatgcaagtcgagcgaacagataaggagcttgctcctttgacgttagcggcggacgggtgagtaacacgtggataacctacctataagactgggataacttcgggaaaccggagctaataccggataacatattgaaccgcatggttcaatagtgaaaggcggctttgctgtcacttatagatggatccgcgccgtattagctagttggtaaggtaacggcttaccaaggcaacgatacgtagccgacctgagagggtgatcggccacactggaactgagacacggtccag

SEQ ID NO: 5 - DNA, 308 bp, Cutibacterium acnes
  source 1..308: mol_type = genomic DNA
gacgaacgctggcggcgtgcttaacacatgcaagtcgaacggaaaggccctgcttttgtggggtgctcgagtggcgaacgggtgagtaacacgtgagtaacctgcccttgactttgggataacttcaggaaactggggctaataccggataggagctcctgctgcatggtgggggttggaaagtttcggcggttggggatggactcgcggcttatcagcttgttggtggggtagtggcttaccaaggctttgacgggtagccggcctgagagggtgaccggccacattgggactgagatacggcccag

SEQ ID NO: 6 - DNA, 304 bp, Corynebacterium tuberculostearicum
  source 1..304: mol_type = genomic DNA
gacgaacgctggcggcgtgcttaacacatgcaagtcgaacggaaaggccctgcttgcagggtactcgagtggcgaacgggtgagtaacacgtgggtgatctgccctgcacttcgggataagcctgggaaactgggtctaataccggataggagccatttttagtgtgatggttggaaagttttttcggtgtaggatgagctcgcggcctatcagcttgttggtggggtaatggcctaccaaggcggcgacgggtagccggcctgagagggtggacggccacattgggactgagatacggcccag

SEQ ID NO: 7 - DNA, 317 bp, Staphylococcus capitis
  source 1..317: mol_type = genomic DNA
gatgaacgctggcggcgtgcctaatacatgcaagtcgagcgaacagacgaggagcttgctcctctgacgttagcggcggacgggtgagtaacacgtggataacctacctataagactgggataacttcgggaaaccggagctaataccggataacatgttgaaccgcatggttcaacagtgaaagacggtcttgctgtcacttatagatggatccgcgccgcattagctagttggtaaggtaacggcttaccaaggcaacgatgcgtagccgacctgagagggtgatcggccacactggaactgagacacggtccag

SEQ ID NO: 8 - DNA, 317 bp, Staphylococcus epidermidis
  source 1..317: mol_type = genomic DNA
gatgaacgctggcggcgtgcctaatacatgcaagtcgagcgaacagacgaggagcttgctcctctgacgttagcggcggacgggtgagtaacacgtggataacctacctataagactgggataacttcgggaaaccggagctaataccggataatatattgaaccgcatggttcaatagtgaaagacggttttgctgtcacttatagatggatccgcgccgcattagctagttggtaaggtaacggcttaccaaggcaacgatgcgtagccgacctgagagggtgatcggccacactggaactgagacacggtccag

SEQ ID NO: 9 - DNA, 300 bp, Moraxella osloensis
  source 1..300: mol_type = genomic DNA
attgaacgctggcggcaggcttaacacatgcaagtcgaacgatgactctctagcttgctagagatgattagtggcggacgggtgagtaacatttaggaatctacctagtagtgggggatagctcggggaaactcgaattaataccgcatacgacctacgggtgaaagggggcgcaagctcttgctattagatgagcctaaatcagattagctagttggtggggtaaaggcccaccaaggcgacgatctgtaactggtctgagaggatgatcagtcacaccggaactgagacacggtccgg

SEQ ID NO: 10 - DNA, 309 bp, Dermacoccus nishinomiyaensis
  source 1..309: mol_type = genomic DNA
gacgaacgctggcggcgtgcttaacacatgcaagtcgaacgatgaagcaccagcttgctggtgtggattagtggcgaacgggtgagtaacacgtgagtaacctgcccctcactctgggataagcctgggaaactgggtctaatactggatacgaccgatctccgcatggagtgttggtggaaagtttttgtggtgggggatggactcgcggcctatcagcttgttggtggggtaatggcctaccaaggcgacgacgggtagccggcctgagagggcgaccggccacactgggactgagacacggcccag

SEQ ID NO: 11 - DNA, 306 bp, Micrococcus luteus
  source 1..306: mol_type = genomic DNA
gatgaacgctggcggcgtgcttaacacatgcaagtcgaacgatgaagcccagcttgctgggtggattagtggcgaacgggtgagtaacacgtgagtaacctgcccttaactctgggataagcctgggaaactgggtctaataccggataggagcgtccaccgcatggtgggtgttggaaagatttatcggttttggatggactcgcggcctatcagcttgttggtgaggtaatggctcaccaaggcgacgacgggtagccggcctgagagggtgaccggccacactgggactgagacacggcccag

SEQ ID NO: 12 - DNA, 280 bp, Enhydrobacter aerosaccus
  source 1..280: mol_type = genomic DNA
aacgaacgctggcggcaggcttaacacatgcaagtcgaacgcgtgtagcaatacacgagtggcgcacgggtgagtaacgcgtggatatctgccttttggttcggaataaccccgggaaactggggctaataccggatggttcctacgggataaagatttatcgccaaaagatgagtccgcgtccgattagctagttggtggggtaacggcctaccaaggcgacgatcggtagctggtctgagaggacgatcagccacactgggactgagacacggcccag

SEQ ID NO: 13 - DNA, 323 bp, Finegoldia magna
  source 1..323: mol_type = genomic DNA
gacgaacgctggcggcgtgcttaacacatgcaagtcgaacgggatttagtagacagaagcttcggtggaagattactaatgagagtggcgaacgggtgagtaacgcgtgagcaacctgcctatgacagtgggatagcctcgggaaaccgggattaataccgcataaaatcgtagaaacacatgttttaacggtcaaagatttatcggtcatagatgggctcgcgtctgattagctagttggtgagataacagcccaccaaggcgacgatcagtagccggtctgagaggatgaacggccacattggaactgagacacggtccaa

SEQ ID NO: 14 - DNA, 317 bp, Staphylococcus aureus
  source 1..317: mol_type = genomic DNA
gatgaacgctggcggcgtgcctaatacatgcaagtcgagcgaacggacgagaagcttgcttctctgatgttagcggcggacgggtgagtaacacgtggataacctacctataagactgggataacttcgggaaaccggagctaataccggataatattttgaaccgcatggttcaaaagtgaaagacggtcttgctgtcacttatagatggatccgcgctgcattagctagttggtaaggtaacggcttaccaaggcaacgatgcatagccgacctgagagggtgatcggccacactggaactgagacacggtccag

SEQ ID NO: 15 - DNA, 317 bp, Staphylococcus hominis
  source 1..317: mol_type = genomic DNA
gatgaacgctggcggcgtgcctaatacatgcaagtcgagcgaacagacgaggagcttgctcctttgacgttagcggcggacgggtgagtaacacgtgggtaacctacctataagactgggataacttcgggaaaccggagctaataccggataatatttcgaaccgcatggttcgatagtgaaagatggctttgctatcacttatagatggacctgcgccgtattagctagttggtaaggtaacggcttaccaaggcaacgatacgtagccgacctgagagggtgatcggccacactggaactgagacacggtccag